European Patent Specification EP 3 917 995 B1, published November 13, 2024. Title: PROTEIN-COATED MATERIALS. Applicant: MODERN MEADOW, INC. The sequence listing filed with the application follows.

SEQUENCE LISTING (1 sequence)

SEQ ID NO: 1 - protein, 1248 aa, Artificial Sequence
  Col3 alpha chain
MFSPILSLEIILALATLQSVFAQQEAVDGGCSHLGQSYADRDVWKPEPCQICVCDSGSVLCDDIICDDQELDCPNPEIPFGECCAVCPQPPTAPTRPPNGQGPQGPKGDPGPPGIPGRNGDPGPPGSPGSPGSPGPPGICESCPTGGQNYSPQYEAYDVKSGVAGGGIAGYPGPAGPPGPPGPPGTSGHPGAPGAPGYQGPPGEPGQAGPAGPPGPPGAIGPSGPAGKDGESGRPGRPGERGFPGPPGMKGPAGMPGFPGMKGHRGFDGRNGEKGETGAPGLKGENGVPGENGAPGPMGPRGAPGERGRPGLPGAAGARGNDGARGSDGQPGPPGPPGTAGFPGSPGAKGEVGPAGSPGSSGAPGQRGEPGPQGHAGAPGPPGPPGSNGSPGGKGEMGPAGIPGAPGLIGARGPPGPPGTNGVPGQRGAAGEPGKNGAKGDPGPRGERGEAGSPGIAGPKGEDGKDGSPGEPGANGLPGAAGERGVPGFRGPAGANGLPGEKGPPGDRGGPGPAGPRGVAGEPGRDGLPGGPGLRGIPGSPGGPGSDGKPGPPGSQGETGRPGPPGSPGPRGQPGVMGFPGPKGNDGAPGKNGERGGPGGPGPQGPAGKNGETGPQGPPGPTGPSGDKGDTGPPGPQGLQGLPGTSGPPGENGKPGEPGPKGEAGAPGIPGGKGDSGAPGERGPPGAGGPPGPRGGAGPPGPEGGKGAAGPPGPPGSAGTPGLQGMPGERGGPGGPGPKGDKGEPGSSGVDGAPGKDGPRGPTGPIGPPGPAGQPGDKGESGAPGVPGIAGPRGGPGERGEQGPPGPAGFPGAPGQNGEPGAKGERGAPGEKGEGGPPGAAGPAGGSGPAGPPGPQGVKGERGSPGGPGAAGFPGGRGPPGPPGSNGNPGPPGSSGAPGKDGPPGPPGSNGAPGSPGISGPKGDSGPPGERGAPGPQGPPGAPGPLGIAGLTGARGLAGPPGMPGARGSPGPQGIKGENGKPGPSGQNGERGPPGPQGLPGLAGTAGEPGRDGNPGSDGLPGRDGAPGAKGDRGENGSPGAPGAPGHPGPPGPVGPAGKSGDRGETGPAGPSGAPGPAGSRGPPGPQGPRGDKGETGERGAMGIKGHRGFPGNPGAPGSPGPAGHQGAVGSPGPAGPRGPVGPSGPPGKDGASGHPGPIGPPGPRGNRGERGSEGSPGHPGQPGPPGPPGAPGPCCGAGGVAAIAGVGAEKAGGFAPYYGDGYIPEAPRDGQAYVRKDGEWVLLSTFL